European Patent Application EP 4 467 136 A2, published November 27, 2024. Title: Antagonists of Cav2.3 R-type calcium channels for the treatment of neurodegenerative diseases. Applicant: Lario Therapeutics Ltd. The sequence listing filed with the application follows.

SEQUENCE LISTING (56 sequences)

SEQ ID NO: 1 - DNA, 28 bp, synthetic construct
  misc_feature 1..28: note = Synthetic
  source 1..28: mol_type = other DNA
ccttgtcggttcctgctctggtccgagt

SEQ ID NO: 2 - DNA, 28 bp, synthetic construct
  misc_feature 1..28: note = Synthetic
  source 1..28: mol_type = other DNA
ccgccggccccgaggccgggacgggggt

SEQ ID NO: 3 - DNA, 20 bp, synthetic construct
  misc_feature 1..20: note = Synthetic
  source 1..20: mol_type = other DNA
tcaccactctgctgcagttc

SEQ ID NO: 4 - DNA, 20 bp, synthetic construct
  misc_feature 1..20: note = Synthetic
  source 1..20: mol_type = other DNA
gacgaaacccacgaagatgt

SEQ ID NO: 5 - DNA, 20 bp, synthetic construct
  misc_feature 1..20: note = Synthetic
  source 1..20: mol_type = other DNA
tcgggactggtctattctgg

SEQ ID NO: 6 - DNA, 20 bp, synthetic construct
  misc_feature 1..20: note = Synthetic
  source 1..20: mol_type = other DNA
tacttccccaccagtccttg

SEQ ID NO: 7 - DNA, 21 bp, synthetic construct
  misc_feature 1..21: note = Synthetic
  source 1..21: mol_type = other DNA
ttggatctgcttgtgcccatg

SEQ ID NO: 8 - DNA, 23 bp, synthetic construct
  misc_feature 1..23: note = Synthetic
  source 1..23: mol_type = other DNA
ggaatttgaacgcttatcccgaa

SEQ ID NO: 9 - DNA, 21 bp, synthetic construct
  misc_feature 1..21: note = Synthetic
  source 1..21: mol_type = other DNA
ccgagcatggggaaatccaac

SEQ ID NO: 10 - DNA, 22 bp, synthetic construct
  misc_feature 1..22: note = Synthetic
  source 1..22: mol_type = other DNA
tcatggcaaagatccggtccac

SEQ ID NO: 11 - DNA, 19 bp, synthetic construct
  misc_feature 1..19: note = Synthetic
  source 1..19: mol_type = other DNA
cgcactctcaaactagccg

SEQ ID NO: 12 - DNA, 22 bp, synthetic construct
  misc_feature 1..22: note = Synthetic
  source 1..22: mol_type = other DNA
cagcctacttctttatagcgca

SEQ ID NO: 13 - DNA, 21 bp, synthetic construct
  misc_feature 1..21: note = Synthetic
  source 1..21: mol_type = other DNA
gagatctggcttcatttcgac

SEQ ID NO: 14 - DNA, 21 bp, synthetic construct
  misc_feature 1..21: note = Synthetic
  source 1..21: mol_type = other DNA
agttccagctttccgtcatta

SEQ ID NO: 15 - DNA, 20 bp, synthetic construct
  misc_feature 1..20: note = Synthetic
  source 1..20: mol_type = other DNA
agaacaacctggctgcgtat

SEQ ID NO: 16 - DNA, 20 bp, synthetic construct
  misc_feature 1..20: note = Synthetic
  source 1..20: mol_type = other DNA
gctcctgcttcgagtcctta

SEQ ID NO: 17 - DNA, 20 bp, synthetic construct
  misc_feature 1..20: note = Synthetic
  source 1..20: mol_type = other DNA
agaaaggttgaatcgctgga

SEQ ID NO: 18 - DNA, 20 bp, synthetic construct
  misc_feature 1..20: note = Synthetic
  source 1..20: mol_type = other DNA
ccagggctagcttaacgttg

SEQ ID NO: 19 - DNA, 20 bp, synthetic construct
  misc_feature 1..20: note = Synthetic
  source 1..20: mol_type = other DNA
catacgcagacagcacgttt

SEQ ID NO: 20 - DNA, 20 bp, synthetic construct
  misc_feature 1..20: note = Synthetic
  source 1..20: mol_type = other DNA
aaaagattccatcgccagag

SEQ ID NO: 21 - DNA, 20 bp, synthetic construct
  misc_feature 1..20: note = Synthetic
  source 1..20: mol_type = other DNA
gggatgtcaactacgcgttt

SEQ ID NO: 22 - DNA, 20 bp, synthetic construct
  misc_feature 1..20: note = Synthetic
  source 1..20: mol_type = other DNA
cacaaatacaggggcgatct

SEQ ID NO: 23 - DNA, 20 bp, synthetic construct
  misc_feature 1..20: note = Synthetic
  source 1..20: mol_type = other DNA
tgacatcgactgccaatacc

SEQ ID NO: 24 - DNA, 20 bp, synthetic construct
  misc_feature 1..20: note = Synthetic
  source 1..20: mol_type = other DNA
gggttagagatgaccatccg

SEQ ID NO: 25 - DNA, 20 bp, synthetic construct
  misc_feature 1..20: note = Synthetic
  source 1..20: mol_type = other DNA
catatgaaattgcacccgtg

SEQ ID NO: 26 - DNA, 20 bp, synthetic construct
  misc_feature 1..20: note = Synthetic
  source 1..20: mol_type = other DNA
cggtgtcataggagacgtca

SEQ ID NO: 27 - DNA, 20 bp, synthetic construct
  misc_feature 1..20: note = Synthetic
  source 1..20: mol_type = other DNA
cacctggagtactttgtgcg

SEQ ID NO: 28 - DNA, 20 bp, synthetic construct
  misc_feature 1..20: note = Synthetic
  source 1..20: mol_type = other DNA
cctgtgggtggtaccctatg

SEQ ID NO: 29 - DNA, 20 bp, synthetic construct
  misc_feature 1..20: note = Synthetic
  source 1..20: mol_type = other DNA
tgcacacagtacatccgtca

SEQ ID NO: 30 - DNA, 20 bp, synthetic construct
  misc_feature 1..20: note = Synthetic
  source 1..20: mol_type = other DNA
tctgacacgaagtacaccgg

SEQ ID NO: 31 - DNA, 23 bp, synthetic construct
  misc_feature 1..23: note = Synthetic
  source 1..23: mol_type = other DNA
ccatctacttcattgtgctcacc

SEQ ID NO: 32 - DNA, 19 bp, synthetic construct
  misc_feature 1..19: note = Synthetic
  source 1..19: mol_type = other DNA
ccccttcatccagactccg

SEQ ID NO: 33 - DNA, 21 bp, synthetic construct
  misc_feature 1..21: note = Synthetic
  source 1..21: mol_type = other DNA
gacagcagctggaagaacaga

SEQ ID NO: 34 - DNA, 23 bp, synthetic construct
  misc_feature 1..23: note = Synthetic
  source 1..23: mol_type = other DNA
gatggagctctcacttagggaac

SEQ ID NO: 35 - DNA, 18 bp, synthetic construct
  misc_feature 1..18: note = Synthetic
  source 1..18: mol_type = other DNA
ggaggtcagcccgatgtc

SEQ ID NO: 36 - DNA, 18 bp, synthetic construct
  misc_feature 1..18: note = Synthetic
  source 1..18: mol_type = other DNA
gggctcctctggttgtcc

SEQ ID NO: 37 - DNA, 21 bp, synthetic construct
  misc_feature 1..21: note = Synthetic
  source 1..21: mol_type = other DNA
ctgagtggtcggagtggatac

SEQ ID NO: 38 - DNA, 21 bp, synthetic construct
  misc_feature 1..21: note = Synthetic
  source 1..21: mol_type = other DNA
agagaggaggtgctttcgttc

SEQ ID NO: 39 - DNA, 18 bp, synthetic construct
  misc_feature 1..18: note = Synthetic
  source 1..18: mol_type = other DNA
accactcaaggatgctgc

SEQ ID NO: 40 - DNA, 20 bp, synthetic construct
  misc_feature 1..20: note = Synthetic
  source 1..20: mol_type = other DNA
cgagctttcagagccaacct

SEQ ID NO: 41 - DNA, 23 bp, synthetic construct
  misc_feature 1..23: note = Synthetic
  source 1..23: mol_type = other DNA
gcttgacagcatctccatttcca

SEQ ID NO: 42 - DNA, 18 bp, synthetic construct
  misc_feature 1..18: note = Synthetic
  source 1..18: mol_type = other DNA
cattctccgcctgttcac

SEQ ID NO: 43 - DNA, 25 bp, synthetic construct
  misc_feature 1..25: note = Synthetic
  source 1..25: mol_type = other DNA
ctctgcaccgttatcatgaagtcta

SEQ ID NO: 44 - DNA, 14 bp, synthetic construct
  misc_feature 1..14: note = Synthetic
  source 1..14: mol_type = other DNA
tcggcgggcagcat

SEQ ID NO: 45 - DNA, 25 bp, synthetic construct
  misc_feature 1..25: note = Synthetic
  source 1..25: mol_type = other DNA
tcgaagggtggccagagctgctgta

SEQ ID NO: 46 - DNA, 25 bp, synthetic construct
  misc_feature 1..25: note = Synthetic
  source 1..25: mol_type = other DNA
tccctccagctggtgatgatgaggt

SEQ ID NO: 47 - DNA, 25 bp, synthetic construct
  misc_feature 1..25: note = Synthetic
  source 1..25: mol_type = other DNA
ttctggcctgagtggtcggagtgga

SEQ ID NO: 48 - DNA, 25 bp, synthetic construct
  misc_feature 1..25: note = Synthetic
  source 1..25: mol_type = other DNA
cgagaacaaggatggcaggattgag

SEQ ID NO: 49 - DNA, 25 bp, synthetic construct
  misc_feature 1..25: note = Synthetic
  source 1..25: mol_type = other DNA
cttcttctgctccttcttgatgctc

SEQ ID NO: 50 - DNA, 25 bp, synthetic construct
  misc_feature 1..25: note = Synthetic
  source 1..25: mol_type = other DNA
tacggtgggccttcaagctctacga

SEQ ID NO: 51 - DNA, 24 bp, synthetic construct
  misc_feature 1..24: note = Synthetic
  source 1..24: mol_type = other DNA
ccatcaccctctacatcaccgccc

SEQ ID NO: 52 - DNA, 20 bp, synthetic construct
  misc_feature 1..20: note = Synthetic
  source 1..20: mol_type = other DNA
ccctaaaacccgccacatct

SEQ ID NO: 53 - DNA, 21 bp, synthetic construct
  misc_feature 1..21: note = Synthetic
  source 1..21: mol_type = other DNA
gagcgatggtgagagctaggt

SEQ ID NO: 54 - DNA, 28 bp, synthetic construct
  misc_feature 1..28: note = Synthetic
  source 1..28: mol_type = other DNA
ccgacatcattaccgggttttcctcttg

SEQ ID NO: 55 - DNA, 23 bp, synthetic construct
  misc_feature 1..23: note = Synthetic
  source 1..23: mol_type = other DNA
ccattctcctcctatccctcaac

SEQ ID NO: 56 - DNA, 31 bp, synthetic construct
  misc_feature 1..31: note = Synthetic
  source 1..31: mol_type = other DNA
cacaatctgatgttttggttaaactatattt